European Patent Specification EP 3 230 309 B1, published March 29, 2023. Title: METHODS OF PRODUCING LONG ACTING CTP-MODIFIED GROWTH HORMONE POLYPEPTIDES. Applicant: OPKO Biologics Ltd HERSHKOVITZ, Oren MOSCHCOVICH, Laura. The sequence listing filed with the application follows.

SEQUENCE LISTING (17 sequences)

SEQ ID NO: 1 - protein, 33 aa, Artificial Sequence
  Human origin - amino acid
DPRFQDSSSSKAPPPSLPSPSRLPGPSDTPILQ

SEQ ID NO: 2 - protein, 28 aa, Artificial Sequence
  Human origin - amino acid
SSSSKAPPPSLPSPSRLPGPSDTPILPQ

SEQ ID NO: 3 - protein, 12 aa, Artificial Sequence
  Human origin - amino acid
SSSSKAPPPSLP

SEQ ID NO: 4 - protein, 301 aa, Artificial Sequence
  Human origin - amino acid
MATGSRTSLLLAFGLLCLPWLQEGSASSSSKAPPPSLPSPSRLPGPSDTPILPQFPTIPLSRLFDNAMLRAHRLHQLAFDTYQEFEEAYIPKEQKYSFLQNPQTSLCFSESIPTPSNREETQQKSNLELLRISLLLIQSWLEPVQFLRSVFANSLVYGASDSNVYDLLKDLEEGIQTLMGRLEDGSPRTGQIFKQTYSKFDTNSHNDDALLKNYGLLYCFRKDMDKVETFLRIVQCRSVEGSCGFSSSSKAPPPSLPSPSRLPGPSDTPILPQSSSSKAPPPSLPSPSRLPGPSDTPILPQ

SEQ ID NO: 5 - protein, 217 aa, Homo sapiens
MATGSRTSLLLAFGLLCLPWLQEGSAFPTIPLSRLFDNAMLRAHRLHQLAFDTYQEFEEAYIPKEQKYSFLQNPQTSLCFSESIPTPSNREETQQKSNLELLRISLLLIQSWLEPVQFLRSVFANSLVYGASDSNVYDLLKDLEEGIQTLMGRLEDGSPRTGQIFKQTYSKFDTNSHNDDALLKNYGLLYCFRKDMDKVETFLRIVQCRSVEGSCGF

SEQ ID NO: 6 - protein, 26 aa, Artificial Sequence
  Human origin - amino acid
MATGSRTSLLLAFGLLCLPWLQEGSA

SEQ ID NO: 7 - protein, 275 aa, Artificial Sequence
  Human origin - amino acid
SSSSKAPPPSLPSPSRLPGPSDTPILPQFPTIPLSRLFDNAMLRAHRLHQLAFDTYQEFEEAYIPKEQKYSFLQNPQTSLCFSESIPTPSNREETQQKSNLELLRISLLLIQSWLEPVQFLRSVFANSLVYGASDSNVYDLLKDLEEGIQTLMGRLEDGSPRTGQIFKQTYSKFDTNSHNDDALLKNYGLLYCFRKDMDKVETFLRIVQCRSVEGSCGFSSSSKAPPPSLPSPSRLPGPSDTPILPQSSSSKAPPPSLPSPSRLPGPSDTPILPQ

SEQ ID NO: 8 - protein, 191 aa, Homo sapiens [sequence omitted]

SEQ ID NO: 9 - DNA, 903 bp, Artificial Sequence
  Human origin - nucleic acid
atggccaccggcagcaggaccagcctgctgctggccttcggcctgctgtgcctgccatggctgcaggagggcagcgccagctcttcttctaaggctccacccccatctctgcccagccccagcagactgccgggccccagcgacacacccattctgccccagttccccaccatccccctgagcaggctgttcgacaacgccatgctgagggctcacaggctgcaccagctggcctttgacacctaccaggagttcgaggaagcctacatccccaaggagcagaagtacagcttcctgcagaacccccagacctccctgtgcttcagcgagagcatccccacccccagcaacagagaggagacccagcagaagagcaacctggagctgctgaggatctccctgctgctgatccagagctggctggagcccgtgcagttcctgagaagcgtgttcgccaacagcctggtgtacggcgccagcgacagcaacgtgtacgacctgctgaaggacctggaggagggcatccagaccctgatgggccggctggaggacggcagccccaggaccggccagatcttcaagcagacctacagcaagttcgacaccaacagccacaacgacgacgccctgctgaagaactacgggctgctgtactgcttcagaaaggacatggacaaggtggagaccttcctgaggatcgtgcagtgcagaagcgtggagggcagctgcggcttcagctccagcagcaaggcccctcccccgagcctgccctccccaagcaggctgcctgggccctccgacacaccaatcctgccacagagcagctcctctaaggcccctcctccatccctgccatccccctcccggctgcctggcccctctgacacccctatcctgcctcag

SEQ ID NO: 10 - protein, 20 aa, Artificial Sequence
  Human origin - amino acid
LPGPSDTPILPQFPTIPLSR

SEQ ID NO: 11 - protein, 31 aa, Artificial Sequence
  Human origin - amino acid
APPPSLPSPSRLPGPSDTPILPQFPTIPLSR

SEQ ID NO: 12 - protein, 12 aa, Artificial Sequence
  Human origin - amino acid
LPGPSDTPILPQ

SEQ ID NO: 13 - protein, 13 aa, Artificial Sequence
  Human origin - amino acid
SVEGSCGFSSSSK

SEQ ID NO: 14 - protein, 51 aa, Artificial Sequence
  Human origin - amino acid
APPPSLPSPSRLPGPSDTPILPQSSSSKAPPPSLPSPSRLPGPSDTPILPQ

SEQ ID NO: 15 - protein, 36 aa, Artificial Sequence
  Human origin - amino acid
SSSSKAPPPSLPSPSRLPGPSDTPILPQFPTIPLSR

SEQ ID NO: 16 - protein, 23 aa, Artificial Sequence
  Human origin - amino acid
APPPSLPSPSRLPGPSDTPILPQ

SEQ ID NO: 17 - protein, 64 aa, Artificial Sequence
  Human origin - amino acid
SVEGSCGFSSSSKAPPPSLPSPSRLPGPSDTPILPQSSSSKAPPPSLPSPSRLPGPSDTPILPQ